European Patent Application EP 4 420 676 A1, published August 28, 2024. Title: CHIMERIC ANTIGEN RECEPTOR. Applicant: Medizinische Hochschule Hannover. Application EP 23158624.9, filed February 24, 2023. The sequence listing filed with the application follows.

SEQUENCE LISTING (206 sequences)

SEQ ID NO: 1 - protein, 8 aa, synthetic construct
GFTFSSYG

SEQ ID NO: 2 - protein, 8 aa, synthetic construct
ISYDGSNK

SEQ ID NO: 3 - protein, 16 aa, synthetic construct
AKDRGAVAGTDWYFDL

SEQ ID NO: 4 - protein, 6 aa, synthetic construct
SLRSYY

SEQ ID NO: 5 - skipped

SEQ ID NO: 6 - protein, 11 aa, synthetic construct
NSRDSSGNHVV

SEQ ID NO: 7 - protein, 8 aa, synthetic construct
GFTFSSYS

SEQ ID NO: 8 - protein, 7 aa, synthetic construct
ITRGGNT

SEQ ID NO: 9 - protein, 14 aa, synthetic construct
AKDWTMSGINVFDT

SEQ ID NO: 10 - protein, 9 aa, synthetic construct
SSDVGAYNR

SEQ ID NO: 11 - skipped

SEQ ID NO: 12 - protein, 10 aa, synthetic construct
SSSTTSSTYV

SEQ ID NO: 13 - protein, 8 aa, synthetic construct
EFPFSSYA

SEQ ID NO: 14 - protein, 8 aa, synthetic construct
ISSSGGDT

SEQ ID NO: 15 - protein, 8 aa, synthetic construct
AKNWNLDY

SEQ ID NO: 16 - protein, 6 aa, synthetic construct
SLRSYY

SEQ ID NO: 17 - skipped

SEQ ID NO: 18 - protein, 12 aa, synthetic construct
NSRDSSGHHNVL

SEQ ID NO: 19 - protein, 8 aa, synthetic construct
GFTVSSNY

SEQ ID NO: 20 - protein, 7 aa, synthetic construct
IYSGGST

SEQ ID NO: 21 - protein, 9 aa, synthetic construct
ARGWTTFDY

SEQ ID NO: 22 - protein, 6 aa, synthetic construct
QLGDRY

SEQ ID NO: 23 - skipped

SEQ ID NO: 24 - protein, 9 aa, synthetic construct
QTWDNSPVV

SEQ ID NO: 25 - protein, 8 aa, synthetic construct
GFTFSSYG

SEQ ID NO: 26 - protein, 8 aa, synthetic construct
ISYDGSNK

SEQ ID NO: 27 - protein, 16 aa, synthetic construct
AKDLTRSGYPSYYFDY

SEQ ID NO: 28 - protein, 6 aa, synthetic construct
SLRSYY

SEQ ID NO: 29 - skipped

SEQ ID NO: 30 - protein, 11 aa, synthetic construct
NSRGSSGNNWV

SEQ ID NO: 31 - protein, 8 aa, synthetic construct
GFTFSSNA

SEQ ID NO: 32 - protein, 7 aa, synthetic construct
IGTGGTT

SEQ ID NO: 33 - protein, 8 aa, synthetic construct
AKTGQLDY

SEQ ID NO: 34 - protein, 9 aa, synthetic construct
SSDVGGYNY

SEQ ID NO: 35 - skipped

SEQ ID NO: 36 - protein, 11 aa, synthetic construct
AAWDDSLSGWV

SEQ ID NO: 37 - protein, 8 aa, synthetic construct
GFTFSNYA

SEQ ID NO: 38 - protein, 8 aa, synthetic construct
ISGGGDNT

SEQ ID NO: 39 - protein, 17 aa, synthetic construct
AKKQSGGSGWSLWGFDY

SEQ ID NO: 40 - protein, 9 aa, synthetic construct
TGAVTSGYY

SEQ ID NO: 41 - skipped

SEQ ID NO: 42 - protein, 9 aa, synthetic construct
LLYYGGRGV

SEQ ID NO: 43 - protein, 8 aa, synthetic construct
GFTFSSYA

SEQ ID NO: 44 - protein, 8 aa, synthetic construct
ISGSGGST

SEQ ID NO: 45 - protein, 17 aa, synthetic construct
AKNPIQLWSKIKNWFDP

SEQ ID NO: 46 - protein, 9 aa, synthetic construct
AGDVTYGHF

SEQ ID NO: 47 - skipped

SEQ ID NO: 48 - protein, 9 aa, synthetic construct
ALSYFGSMF

SEQ ID NO: 49 - protein, 8 aa, synthetic construct
GFTFSSYG

SEQ ID NO: 50 - protein, 8 aa, synthetic construct
ISYDGSNK

SEQ ID NO: 51 - protein, 16 aa, synthetic construct
AKDLTRSGYPSYYFDY

SEQ ID NO: 52 - protein, 6 aa, synthetic construct
SLRSYY

SEQ ID NO: 53 - skipped

SEQ ID NO: 54 - protein, 10 aa, synthetic construct
NSRDSSGNLV

SEQ ID NO: 55 - protein, 123 aa, synthetic construct
QVQLVQSGGGVVQPGRSLRLSCAASGFTFSSYGMHWVRQAPGKGLEWVAVISYDGSNKYYADSVKGRFTISRDNSKNTLYLQMNSLRAEDTAVYYCAKDRGAVAGTDWYFDLWGRGTLVTVSS

SEQ ID NO: 56 - protein, 108 aa, synthetic construct
SSELTQDPAVSVALGQTVRITCQGDSLRSYYASWYQQKPGQAPVLVIYGKNNRPSGIPDRFSGSSSGNTASLTITGAQAEDEADYYCNSRDSSGNHVVFGGGTKLTVL

SEQ ID NO: 57 - protein, 120 aa, synthetic construct
QVQLVQSGGGLVQPGGSLRLSCAASGFTFSSYSMSWVRQAPGKGLEWVLGITRGGNTFYADSVTGRFTISRDISKNTVFLQMDSLRVEDTAIYYCAKDWTMSGINVFDTWGQGTLVTVSS

SEQ ID NO: 58 - protein, 110 aa, synthetic construct
QAVLTQPPSVSGSPGQSVTISCTGTSSDVGAYNRVSWYQQPPGTAPKLMIYEVNNRPSGVPDRFSGSKSGNTASLTISGLQAEDEADYYCSSSTTSSTYVFGTGTKVTVL

SEQ ID NO: 59 - protein, 115 aa, synthetic construct
EVQLQQSGGGLVQPGGSLRLSCAASEFPFSSYAMSWVRQAPGKGLAWVSAISSSGGDTYYADSVKGRFTISRDNSKNTLYLQMNSLRAEDTAVYYCAKNWNLDYWGQGTLVTVSS

SEQ ID NO: 60 - protein, 109 aa, synthetic construct
SSELTQDPAVSVALGQTVMITCQGHSLRSYYASWYQQKPGQAPLLVIYGDNRRPSGIPDRFSGSNSGNTASLTITGTQAEDEADYYCNSRDSSGHHNVLFGGGTKLTVL

SEQ ID NO: 61 - protein, 115 aa, synthetic construct
EVQLVESGGGLVQPGGSLRLSCAASGFTVSSNYMSWVRQAPGKGLEWVSVIYSGGSTYYADSVKGRFTISRDNAKNSLYLQMNSLRAEDTAVYYCARGWTTFDYWGQGTLVTVSS

SEQ ID NO: 62 - protein, 106 aa, synthetic construct
QAVLTQPPSLSVSPRQTVTITCSGDQLGDRYVSWYQQKPGQSPMLVIYQDDRRPSGVPERFSGSNSGNTATLTIGGTQAMDQADYYCQTWDNSPVVFGGGTKLTVL

SEQ ID NO: 63 - protein, 123 aa, synthetic construct
EVQLVQSGGGVVQPGRSLRLSCAASGFTFSSYGMHWVRQAPGKGLEWVAVISYDGSNKYYADSVKGRFTISRDNSKNTLYLQMNSLRAEDTAVYYCAKDLTRSGYPSYYFDYWGQGTLVTVSS

SEQ ID NO: 64 - protein, 108 aa, synthetic construct
SSELTQDPAVSVALGQTVRITCQGDSLRSYYASWYQQKPGQAPVLVIYGKNNRPSGIPDRFSGSSSGNTASLTITGAQAEDEADYYCNSRGSSGNNWVFGGGTKLTVL

SEQ ID NO: 65 - protein, 114 aa, synthetic construct
QVQLVESGGGLVQPGGSLRLSCAASGFTFSSNAMSWVRQAPGKGLEWVSAIGTGGTTYYADSVKGRFTISRDNSKNTLYLQMNSLRAEDTAVYYCAKTGQLDYWGQGTLVTVSS

SEQ ID NO: 66 - protein, 111 aa, synthetic construct
QSALTQPASVSGSPGQSITISCTGTSSDVGGYNYVSWFQQHPDKAPKLMIYDVSNRPSGVSNRFSGSKSGTSASLAISGLRSEDEADYYCAAWDDSLSGWVFGGGTKLTVL

SEQ ID NO: 67 - protein, 124 aa, synthetic construct
QVQLVQSGGGLVQPGGSLRLSCAASGFTFSNYAMSWVRQAPGKGLEWVSGISGGGDNTYYTDSVKGRFTISRDNSKNTLYLQMNSLTAEDTALYYCAKKQSGGSGWSLWGFDYWGQGTLVTVSS

SEQ ID NO: 68 - protein, 109 aa, synthetic construct
QAVVTQEPSLTVSPGGTVTLTCASSTGAVTSGYYPSWFQQKPGQAPRPLIYNTNNKHSWSPARFSGSLLGGKAALTLSGVQPEDEADYYCLLYYGGRGVFGGGTRLTVL

SEQ ID NO: 69 - protein, 124 aa, synthetic construct
EVQLLESGGGLVQPGGSLRLSCAASGFTFSSYAMSWVRQAPGKGLEWVSAISGSGGSTYYADSVKGRFTISRDNSKNTLYLQMNSLRAEDTAVYYCAKNPIQLWSKIKNWFDPWGQGTLVTVSS

SEQ ID NO: 70 - protein, 109 aa, synthetic construct
QAVVTQEPSLSVSPGGTVSLTCGSSAGDVTYGHFPYWYQQKPGQAPRMLIYDVNNRASWTPARFSGSLVGGKAALTLSGAQPGDEADYYCALSYFGSMFFGGGTKLTVL

SEQ ID NO: 71 - protein, 123 aa, synthetic construct; identical to SEQ ID NO: 63

SEQ ID NO: 72 - protein, 107 aa, synthetic construct
SSELTQDPAVSVALGRTVRITCQGDSLRSYYASWYQQKPGQAPVLVIYGKNNRPSGIPDRFSGSSSGNTASLTITGAQAEDEADYYCNSRDSSGNLVFGGGTKLTVL

SEQ ID NO: 73 - DNA, 370 bp, synthetic construct
  source 1..370: mol_type = other DNA
caggtgcagctggtgcagtctgggggaggcgtggtccagcctgggaggtccctgagactctcctgtgcagcctctggattcaccttcagtagctatggcatgcactgggtccgccaggctccaggcaaggggctggagtgggtggcagttatatcatatgatggaagtaataaatactatgcagactccgtgaagggccgattcaccatctccagagacaattccaagaacacgctgtatctgcaaatgaacagcctgagagctgaggacacggctgtgtattactgtgcgaaagatcggggagcagtggctgggactgactggtacttcgatctctggggccgtggcaccctggtcactgtctcctcag

SEQ ID NO: 74 - DNA, 325 bp, synthetic construct
  source 1..325: mol_type = other DNA
tcttctgagctgactcaggaccctgctgtgtctgtggccttgggacagacagtcaggatcacatgccaaggagacagcctcagaagctattatgcaagctggtaccagcagaagccaggacaggcccctgtacttgtcatctatggtaaaaacaaccggccctcagggatcccagaccgattctctggctccagctcaggaaacacagcttccttgaccatcactggggctcaggcggaagatgaggctgactattactgtaactcccgggacagcagtggtaaccatgtggtattcggcggagggaccaagctgaccgtcctag

SEQ ID NO: 75 - DNA, 361 bp, synthetic construct
  source 1..361: mol_type = other DNA
caggtccagctggtgcaatctgggggaggcttggtacagccgggggggtccctgagactctcctgtgcagcctctggattcaccttcagtagctatagcatgagctgggtccgccaggccccagggaaggggctggagtgggtcttaggtattactcgtggtggtaacacattctacgcagactccgtgacgggccggttcaccatctccagagacatttccaagaacacggtgtttctgcaaatggacagcctgagagtcgaggacacggccatttattactgtgcgaaagactggaccatgagtggaatcaacgtcttcgacacctggggccaggggaccctggtcaccgtctcctccg

SEQ ID NO: 76 - DNA, 331 bp, synthetic construct
  source 1..331: mol_type = other DNA
caggcagtgctgactcagccaccctccgtgtccgggtctcctggacagtcagtcaccatctcctgcactggaaccagcagtgacgttggtgcttataaccgtgtctcctggtaccagcagcccccaggcacagcccccaaacttatgatttatgaggtcaataatcggccctcaggggtccctgatcgcttctctgggtccaagtctggcaacacggcctccctgaccatctctgggctccaggctgaggacgaggctgattattactgcagctcatctacaaccagtagcacttatgtcttcggaactgggaccaaggtcaccgtcctag

SEQ ID NO: 77 - DNA, 346 bp, synthetic construct
  source 1..346: mol_type = other DNA
gaagtgcagctacagcagtccgggggaggcttggtacagcctggggggtccctgagactctcctgtgcagcctctgaattcccctttagcagctatgccatgagctgggtccgccaggctccagggaaggggctggcgtgggtctcagctattagtagtagtggtggtgacacatactacgcagactccgtgaagggccggttcaccatctccagagacaattccaagaacacgctgtatctgcaaatgaacagcctgagagccgaggacacggccgtatattactgtgcgaaaaactggaaccttgactactggggccagggaaccctggtcaccgtctcctcag

SEQ ID NO: 78 - DNA, 327 bp, synthetic construct
  source 1..327: mol_type = other DNA
tcttctgagctgactcaggaccctgctgtgtctgtggccttgggacagacagtcatgataacatgccaaggacacagcctccgaagctattatgcaagctggtaccagcagaagccaggacaggcccctctacttgtcatctatggtgacaacaggcggccctcagggatcccagaccgattctctggctccaactcaggaaacacagcttccttgaccatcactgggactcaggcggaagatgaggctgactactattgtaattctcgggacagtagtggtcaccataatgtgctattcggcggggggaccaagctgaccgtccta

SEQ ID NO: 79 - DNA, 346 bp, synthetic construct
  source 1..346: mol_type = other DNA
gaggtgcagctggtggagtctgggggaggcttggtccagcctggggggtccctgagactctcctgtgcagcctctggattcaccgtcagtagcaactacatgagctgggtccgccaggctccagggaaggggctggagtgggtctcagttatttatagcggtggtagcacatactacgcagactccgtgaagggccgattcaccatctccagagacaacgccaagaactcactgtatctgcaaatgaacagcctgagagctgaggacacggctgtgtattactgtgcgaggggttggacgacttttgactactggggccagggaaccctggtcaccgtctcctcag

SEQ ID NO: 80 - DNA, 319 bp, synthetic construct
  source 1..319: mol_type = other DNA
caggctgtgctgactcagcccccctcactgtctgtgtccccaagacagacagtcaccatcacctgctctggagatcaactgggagatagatatgtttcctggtatcagcagaagccaggccagtcccctatgttggtcatctatcaagatgacaggcggccctcaggggtccctgagcgattctctggctccaactctgggaacacagccactctgaccatcggcgggacccaggctatggatcaggctgattattattgtcaaacgtgggacaacagtcctgtggtgtttggcggggggaccaaattgaccgtcctag

SEQ ID NO: 81 - DNA, 370 bp, synthetic construct
  source 1..370: mol_type = other DNA
gaagtgcagctggtgcagtctgggggaggcgtggtccagcctgggaggtccctgagactctcctgtgcagcctctggattcaccttcagtagctatggcatgcactgggtccgccaggctccaggcaaggggctggagtgggtggcagttatttcatatgatggaagtaataaatactatgcagactccgtgaagggccgattcaccatctccagagacaattccaagaacacgctgtatctgcaaatgaacagcctgagagctgaggacacggctgtgtattattgtgcgaaagatcttacccgaagtggttatccttcctactactttgactactggggccagggaaccctggtcaccgtctcctcag

SEQ ID NO: 82 - DNA, 325 bp, synthetic construct
  source 1..325: mol_type = other DNA
tcttctgagctgactcaggaccctgctgtgtctgtggccttgggacagacagtcaggatcacatgccaaggagacagcctcagaagctattatgcaagctggtaccagcagaagccaggacaggcccctgtacttgtcatctatggtaaaaacaaccggccctcagggatcccagaccgattctctggctccagctcaggaaacacagcttccttgaccatcactggggctcaggcggaagatgaggctgactattactgtaactcccggggcagcagtggtaacaattgggtgttcggcggagggaccaagctgaccgtcctag

SEQ ID NO: 83 - DNA, 343 bp, synthetic construct
  source 1..343: mol_type = other DNA
caagtgcagctggtggagtctgggggaggcttggtacagcctggggggtccctgagactctcctgtgcagcctctggattcacctttagcagcaatgccatgagttgggtccgccaggctccagggaaggggctggagtgggtctcagctattggtactggtggtaccacatactacgcagactccgtgaagggccggttcaccatctccagagacaattccaagaacacgctgtatctgcaaatgaacagcctgagagccgaggacacggccgtatattactgtgcgaaaacgggccaacttgactactggggccagggaaccctggtcaccgtctcctcag

SEQ ID NO: 84 - DNA, 334 bp, synthetic construct
  source 1..334: mol_type = other DNA
cagtctgccctgactcagcctgcctccgtgtctgggtctcctggacagtcgatcaccatctcctgcactggaaccagcagtgacgttggtggttataactatgtctcctggttccaacagcacccagacaaagcccccaaactcatgatttatgatgtcagtaatcggccctcaggggtttctaatcgcttctctggctccaagtctggcacctcagcctccctggccatcagtgggctccggtccgaggatgaggctgattattactgtgcagcatgggatgacagcctgagtgggtgggtgttcggcggagggaccaagctgaccgtcctag

SEQ ID NO: 85 - DNA, 373 bp, synthetic construct
  source 1..373: mol_type = other DNA
caggtgcagctggtacagtctgggggaggcttagtacagcctggggggtccctgagactctcctgtgcagcctctggattcacctttagtaactatgccatgagctgggtccgccaggctccagggaaggggctggagtgggtctcaggtattagtggtggtggtgataacacatactacacagactccgtgaagggccgcttcaccatctccagagacaattccaagaacacgctgtatctgcaaatgaacagcctgacagccgaggacacggccctatattactgtgcgaaaaaacaaagcggaggtagtggctggtccctctggggattcgactactggggccagggaaccctggtcaccgtctcctcag

SEQ ID NO: 86 - DNA, 327 bp, synthetic construct
  source 1..327: mol_type = other DNA
caggctgtggtgacccaggagccctcactgactgtgtccccaggagggacagtcactctcacctgtgcttccagcactggagcagtcaccagtggttactatccaagctggttccagcagaaacctggacaagcacccaggccactaatttataatacaaacaacaaacactcctggagtcctgcccggttctcaggctccctccttgggggcaaagctgccctgacactgtcaggtgtgcagcctgaggacgaggctgactattactgcctgctctactatggtgggcggggagtattcggcggagggaccaggctgaccgtccta

SEQ ID NO: 87 - DNA, 373 bp, synthetic construct
  source 1..373: mol_type = other DNA
gaggtgcagctgttggagtctgggggaggcttggtacagcctggggggtccctgagactctcctgtgcagcctctggattcacctttagcagctatgccatgagctgggtccgccaggctccagggaaggggctggagtgggtctcagctattagtggtagtggtggtagcacatactacgcagactccgtgaagggccggttcaccatctccagagacaattccaagaacacgctgtatctgcaaatgaacagcctgagagccgaggacacggccgtatattactgtgcgaaaaatcccatacagctatggtctaaaataaagaactggttcgacccctggggccagggaaccctggtcaccgtctcctcag

SEQ ID NO: 88 - DNA, 326 bp, synthetic construct
  source 1..326: mol_type = other DNA
caggctgtggtgactcaagagccctcactaagtgtgtccccaggagggacagtcagtctcacctgtggctccagcgctggagatgtcacctatggtcactttccctactggtaccagcagaagcctggccaagcccccagaatgctcatttatgatgtaaacaacagagcgtcctggacccctgcccggttctcaggctccctcgttgggggcaaggctgccctgaccctttcgggtgcgcagcctggggatgaggctgactattactgcgccctctcctattttggttctatgtttttcggcggagggaccaagctgaccgtcct

SEQ ID NO: 89 - DNA, 369 bp, synthetic construct
  source 1..369: mol_type = other DNA
gaggtgcagctggtgcagtctgggggaggcgtggtccagcctgggaggtccctgagactctcctgtgcagcctctggattcaccttcagtagctatggcatgcactgggtccgccaggctccaggcaaggggctggagtgggtggcagttatttcatatgatggaagtaataaatactatgcagactccgtgaagggccgattcaccatctccagagacaattccaagaacacgctgtatctgcaaatgaacagcctgagagctgaggacacggctgtgtattattgtgcgaaagatcttacccgaagtggttatccttcctactactttgactactggggccagggaaccctggtcaccgtctcctca

SEQ ID NO: 90 - DNA, 321 bp, synthetic construct
  source 1..321: mol_type = other DNA
tcttctgagctgactcaggaccctgctgtgtctgtggccttgggacggacagtcaggatcacatgccaaggagacagcctcagaagctattatgcaagctggtaccagcagaagccaggacaggcccctgtacttgtcatctatggtaaaaacaaccggccctcagggatcccagaccgattctctggctccagctcaggaaacacagcttccttgaccatcactggggctcaggcggaagatgaggctgactattactgtaactcccgggacagcagtggtaacctagtattcggcggagggaccaagctgaccgtccta

SEQ ID NO: 91 - protein, 246 aa, synthetic construct
QVQLVQSGGGVVQPGRSLRLSCAASGFTFSSYGMHWVRQAPGKGLEWVAVISYDGSNKYYADSVKGRFTISRDNSKNTLYLQMNSLRAEDTAVYYCAKDRGAVAGTDWYFDLWGRGTLVTVSSGGGGSGGGGSGGGGSSSELTQDPAVSVALGQTVRITCQGDSLRSYYASWYQQKPGQAPVLVIYGKNNRPSGIPDRFSGSSSGNTASLTITGAQAEDEADYYCNSRDSSGNHVVFGGGTKLTVL

SEQ ID NO: 92 - protein, 245 aa, synthetic construct
QVQLVQSGGGLVQPGGSLRLSCAASGFTFSSYSMSWVRQAPGKGLEWVLGITRGGNTFYADSVTGRFTISRDISKNTVFLQMDSLRVEDTAIYYCAKDWTMSGINVFDTWGQGTLVTVSSGGGGSGGGGSGGGGSQAVLTQPPSVSGSPGQSVTISCTGTSSDVGAYNRVSWYQQPPGTAPKLMIYEVNNRPSGVPDRFSGSKSGNTASLTISGLQAEDEADYYCSSSTTSSTYVFGTGTKVTVL

SEQ ID NO: 93 - protein, 239 aa, synthetic construct
EVQLQQSGGGLVQPGGSLRLSCAASEFPFSSYAMSWVRQAPGKGLAWVSAISSSGGDTYYADSVKGRFTISRDNSKNTLYLQMNSLRAEDTAVYYCAKNWNLDYWGQGTLVTVSSGGGGSGGGGSGGGGSSSELTQDPAVSVALGQTVMITCQGHSLRSYYASWYQQKPGQAPLLVIYGDNRRPSGIPDRFSGSNSGNTASLTITGTQAEDEADYYCNSRDSSGHHNVLFGGGTKLTVL

SEQ ID NO: 94 - protein, 236 aa, synthetic construct
EVQLVESGGGLVQPGGSLRLSCAASGFTVSSNYMSWVRQAPGKGLEWVSVIYSGGSTYYADSVKGRFTISRDNAKNSLYLQMNSLRAEDTAVYYCARGWTTFDYWGQGTLVTVSSGGGGSGGGGSGGGGSQAVLTQPPSLSVSPRQTVTITCSGDQLGDRYVSWYQQKPGQSPMLVIYQDDRRPSGVPERFSGSNSGNTATLTIGGTQAMDQADYYCQTWDNSPVVFGGGTKLTVL

SEQ ID NO: 95 - protein, 246 aa, synthetic construct
EVQLVQSGGGVVQPGRSLRLSCAASGFTFSSYGMHWVRQAPGKGLEWVAVISYDGSNKYYADSVKGRFTISRDNSKNTLYLQMNSLRAEDTAVYYCAKDLTRSGYPSYYFDYWGQGTLVTVSSGGGGSGGGGSGGGGSSSELTQDPAVSVALGQTVRITCQGDSLRSYYASWYQQKPGQAPVLVIYGKNNRPSGIPDRFSGSSSGNTASLTITGAQAEDEADYYCNSRGSSGNNWVFGGGTKLTVL

SEQ ID NO: 96 - protein, 240 aa, synthetic construct
QVQLVESGGGLVQPGGSLRLSCAASGFTFSSNAMSWVRQAPGKGLEWVSAIGTGGTTYYADSVKGRFTISRDNSKNTLYLQMNSLRAEDTAVYYCAKTGQLDYWGQGTLVTVSSGGGGSGGGGSGGGGSQSALTQPASVSGSPGQSITISCTGTSSDVGGYNYVSWFQQHPDKAPKLMIYDVSNRPSGVSNRFSGSKSGTSASLAISGLRSEDEADYYCAAWDDSLSGWVFGGGTKLTVL

SEQ ID NO: 97 - protein, 248 aa, synthetic construct
QVQLVQSGGGLVQPGGSLRLSCAASGFTFSNYAMSWVRQAPGKGLEWVSGISGGGDNTYYTDSVKGRFTISRDNSKNTLYLQMNSLTAEDTALYYCAKKQSGGSGWSLWGFDYWGQGTLVTVSSGGGGSGGGGSGGGGSQAVVTQEPSLTVSPGGTVTLTCASSTGAVTSGYYPSWFQQKPGQAPRPLIYNTNNKHSWSPARFSGSLLGGKAALTLSGVQPEDEADYYCLLYYGGRGVFGGGTRLTVL

SEQ ID NO: 98 - protein, 248 aa, synthetic construct
EVQLLESGGGLVQPGGSLRLSCAASGFTFSSYAMSWVRQAPGKGLEWVSAISGSGGSTYYADSVKGRFTISRDNSKNTLYLQMNSLRAEDTAVYYCAKNPIQLWSKIKNWFDPWGQGTLVTVSSGGGGSGGGGSGGGGSQAVVTQEPSLSVSPGGTVSLTCGSSAGDVTYGHFPYWYQQKPGQAPRMLIYDVNNRASWTPARFSGSLVGGKAALTLSGAQPGDEADYYCALSYFGSMFFGGGTKLTVL

SEQ ID NO: 99 - protein, 245 aa, synthetic construct
EVQLVQSGGGVVQPGRSLRLSCAASGFTFSSYGMHWVRQAPGKGLEWVAVISYDGSNKYYADSVKGRFTISRDNSKNTLYLQMNSLRAEDTAVYYCAKDLTRSGYPSYYFDYWGQGTLVTVSSGGGGSGGGGSGGGGSSSELTQDPAVSVALGRTVRITCQGDSLRSYYASWYQQKPGQAPVLVIYGKNNRPSGIPDRFSGSSSGNTASLTITGAQAEDEADYYCNSRDSSGNLVFGGGTKLTVL

SEQ ID NO: 100 - DNA, 927 bp, synthetic construct
  source 1..927: mol_type = other DNA
atgaaatacctattgcctacggcagccgctggcttgctgctgctggcagctcagccggccatggcccaggtgcagctggtgcagtctgggggaggcgtggtccagcctgggaggtccctgagactctcctgtgcagcctctggattcaccttcagtagctatggcatgcactgggtccgccaggctccaggcaaggggctggagtgggtggcagttatatcatatgatggaagtaataaatactatgcagactccgtgaagggccgattcaccatctccagagacaattccaagaacacgctgtatctgcaaatgaacagcctgagagctgaggacacggctgtgtattactgtgcgaaagatcggggagcagtggctgggactgactggtacttcgatctctggggccgtggcaccctggtcactgtctcctcagggagtgcatccgccccaaagcttgaagaaggtgaattttcagaagcacgcgtatcttctgagctgactcaggaccctgctgtgtctgtggccttgggacagacagtcaggatcacatgccaaggagacagcctcagaagctattatgcaagctggtaccagcagaagccaggacaggcccctgtacttgtcatctatggtaaaaacaaccggccctcagggatcccagaccgattctctggctccagctcaggaaacacagcttccttgaccatcactggggctcaggcggaagatgaggctgactattactgtaactcccgggacagcagtggtaaccatgtggtattcggcggagggaccaagctgaccgtcctaggtcagcccaaggctgccccctcggtcactctgttcccaccctcctctgcggccgcaggttctgaacaaaagctgatctcagaagaagatctatcccatcatcaccatcatcat

SEQ ID NO: 101 - DNA, 924 bp, synthetic construct
  source 1..924: mol_type = other DNA
atgaaatacctattgcctacggcagccgctggcttgctgctgctggcagctcagccggccatggcccaggtccagctggtgcaatctgggggaggcttggtacagccgggggggtccctgagactctcctgtgcagcctctggattcaccttcagtagctatagcatgagctgggtccgccaggccccagggaaggggctggagtgggtcttaggtattactcgtggtggtaacacattctacgcagactccgtgacgggccggttcaccatctccagagacatttccaagaacacggtgtttctgcaaatggacagcctgagagtcgaggacacggccatttattactgtgcgaaagactggaccatgagtggaatcaacgtcttcgacacctggggccaggggaccctggtcaccgtctcctccgggagtgcatccgccccaaagcttgaagaaggtgaattttcagaagcacgcgtacaggcagtgctgactcagccaccctccgtgtccgggtctcctggacagtcagtcaccatctcctgcactggaaccagcagtgacgttggtgcttataaccgtgtctcctggtaccagcagcccccaggcacagcccccaaacttatgatttatgaggtcaataatcggccctcaggggtccctgatcgcttctctgggtccaagtctggcaacacggcctccctgaccatctctgggctccaggctgaggacgaggctgattattactgcagctcatctacaaccagtagcacttatgtcttcggaactgggaccaaggtcaccgtcctaggtcagcccaaggccaaccccactgtcactctgttcccaccctcctctgcggccgcaggttctgaacaaaagctgatctcagaagaagatctatcccatcatcaccatcatcat

SEQ ID NO: 102 - DNA, 906 bp, synthetic construct
  source 1..906: mol_type = other DNA
atgaaatacctattgcctacggcagccgctggcttgctgctgctggcagctcagccggccatggccgaagtgcagctacagcagtccgggggaggcttggtacagcctggggggtccctgagactctcctgtgcagcctctgaattcccctttagcagctatgccatgagctgggtccgccaggctccagggaaggggctggcgtgggtctcagctattagtagtagtggtggtgacacatactacgcagactccgtgaagggccggttcaccatctccagagacaattccaagaacacgctgtatctgcaaatgaacagcctgagagccgaggacacggccgtatattactgtgcgaaaaactggaaccttgactactggggccagggaaccctggtcaccgtctcctcagggagtgcatccgccccaaagcttgaagaaggtgaattttcagaagcacgcgtatcttctgagctgactcaggaccctgctgtgtctgtggccttgggacagacagtcatgataacatgccaaggacacagcctccgaagctattatgcaagctggtaccagcagaagccaggacaggcccctctacttgtcatctatggtgacaacaggcggccctcagggatcccagaccgattctctggctccaactcaggaaacacagcttccttgaccatcactgggactcaggcggaagatgaggctgactactattgtaattctcgggacagtagtggtcaccataatgtgctattcggcggggggaccaagctgaccgtcctaagtcagcccaaggctgccccctcggtcactctgttcccaccctcctctgcggccgcaggttctgaacaaaagctgatctcagaagaagatctatcccatcatcaccatcatcat

SEQ ID NO: 103 - DNA, 897 bp, synthetic construct
  source 1..897: mol_type = other DNA
atgaaatacctattgcctacggcagccgctggcttgctgctgctggcagctcagccggccatggccgaggtgcagctggtggagtctgggggaggcttggtccagcctggggggtccctgagactctcctgtgcagcctctggattcaccgtcagtagcaactacatgagctgggtccgccaggctccagggaaggggctggagtgggtctcagttatttatagcggtggtagcacatactacgcagactccgtgaagggccgattcaccatctccagagacaacgccaagaactcactgtatctgcaaatgaacagcctgagagctgaggacacggctgtgtattactgtgcgaggggttggacgacttttgactactggggccagggaaccctggtcaccgtctcctcagggagtgcatccgccccaaagcttgaagaaggtgaattttcagaagcacgcgtacaggctgtgctgactcagcccccctcactgtctgtgtccccaagacagacagtcaccatcacctgctctggagatcaactgggagatagatatgtttcctggtatcagcagaagccaggccagtcccctatgttggtcatctatcaagatgacaggcggccctcaggggtccctgagcgattctctggctccaactctgggaacacagccactctgaccatcggcgggacccaggctatggatcaggctgattattattgtcaaacgtgggacaacagtcctgtggtgtttggcggggggaccaaattgaccgtcctaggtcagcccaaggctgccccctcggtcactctgttcccaccctcctctgcggccgcaggttctgaacaaaagctgatctcagaagaagatctatcccatcatcaccatcatcat

SEQ ID NO: 104 - DNA, 927 bp, synthetic construct
  source 1..927: mol_type = other DNA
atgaaatacctattgcctacggcagccgctggcttgctgctgctggcagctcagccggccatggccgaagtgcagctggtgcagtctgggggaggcgtggtccagcctgggaggtccctgagactctcctgtgcagcctctggattcaccttcagtagctatggcatgcactgggtccgccaggctccaggcaaggggctggagtgggtggcagttatttcatatgatggaagtaataaatactatgcagactccgtgaagggccgattcaccatctccagagacaattccaagaacacgctgtatctgcaaatgaacagcctgagagctgaggacacggctgtgtattattgtgcgaaagatcttacccgaagtggttatccttcctactactttgactactggggccagggaaccctggtcaccgtctcctcagggagtgcatccgccccaaagcttgaagaaggtgaattttcagaagcacgcgtatcttctgagctgactcaggaccctgctgtgtctgtggccttgggacagacagtcaggatcacatgccaaggagacagcctcagaagctattatgcaagctggtaccagcagaagccaggacaggcccctgtacttgtcatctatggtaaaaacaaccggccctcagggatcccagaccgattctctggctccagctcaggaaacacagcttccttgaccatcactggggctcaggcggaagatgaggctgactattactgtaactcccggggcagcagtggtaacaattgggtgttcggcggagggaccaagctgaccgtcctaggtcagcccaaggctgccccctcggtcactctgttcccgccctcctctgcggccgcaggttctgaacaaaagctgatctcagaagaagatctatcccatcatcaccatcatcat

SEQ ID NO: 105 - DNA, 909 bp, synthetic construct
  source 1..909: mol_type = other DNA
atgaaatacctattgcctacggcagccgctggcttgctgctgctggcagctcagccggccatggcccaagtgcagctggtggagtctgggggaggcttggtacagcctggggggtccctgagactctcctgtgcagcctctggattcacctttagcagcaatgccatgagttgggtccgccaggctccagggaaggggctggagtgggtctcagctattggtactggtggtaccacatactacgcagactccgtgaagggccggttcaccatctccagagacaattccaagaacacgctgtatctgcaaatgaacagcctgagagccgaggacacggccgtatattactgtgcgaaaacgggccaacttgactactggggccagggaaccctggtcaccgtctcctcagggagtgcatccgccccaaagcttgaagaaggtgaattttcagaagcacgcgtacagtctgccctgactcagcctgcctccgtgtctgggtctcctggacagtcgatcaccatctcctgcactggaaccagcagtgacgttggtggttataactatgtctcctggttccaacagcacccagacaaagcccccaaactcatgatttatgatgtcagtaatcggccctcaggggtttctaatcgcttctctggctccaagtctggcacctcagcctccctggccatcagtgggctccggtccgaggatgaggctgattattactgtgcagcatgggatgacagcctgagtgggtgggtgttcggcggagggaccaagctgaccgtcctaggtcagcccaaggctgccccctcggtcactctgttcccaccctcctctgcggccgcaggttctgaacaaaagctgatctcagaagaagatctatcccatcatcaccatcatcat

SEQ ID NO: 106 - DNA, 933 bp, synthetic construct
  source 1..933: mol_type = other DNA
atgaaatacctattgcctacggcagccgctggcttgctgctgctggcagctcagccggccatggcccaggtgcagctggtacagtctgggggaggcttagtacagcctggggggtccctgagactctcctgtgcagcctctggattcacctttagtaactatgccatgagctgggtccgccaggctccagggaaggggctggagtgggtctcaggtattagtggtggtggtgataacacatactacacagactccgtgaagggccgcttcaccatctccagagacaattccaagaacacgctgtatctgcaaatgaacagcctgacagccgaggacacggccctatattactgtgcgaaaaaacaaagcggaggtagtggctggtccctctggggattcgactactggggccagggaaccctggtcaccgtctcctcagggagtgcatccgccctaaagcttgaagaaggtgaattttcagaagcacgcgtacaggctgtggtgacccaggagccctcactgactgtgtccccaggagggacagtcactctcacctgtgcttccagcactggagcagtcaccagtggttactatccaagctggttccagcagaaacctggacaagcacccaggccactaatttataatacaaacaacaaacactcctggagtcctgcccggttctcaggctccctccttgggggcaaagctgccctgacactgtcaggtgtgcagcctgaggacgaggctgactattactgcctgctctactatggtgggcggggagtattcggcggagggaccaggctgaccgtcctaagtcagcccaaggctgccccctcggtcactctgttcccaccctcctctgcggccgcaggttctgaacaaaagctgatctcagaagaagatctatcccatcatcaccatcatcat

SEQ ID NO: 107 - DNA, 933 bp, synthetic construct
  source 1..933: mol_type = other DNA
atgaaatacctattgcctacggcagccgctggcttgctgctgctggcagctcagccggccatggccgaggtgcagctgttggagtctgggggaggcttggtacagcctggggggtccctgagactctcctgtgcagcctctggattcacctttagcagctatgccatgagctgggtccgccaggctccagggaaggggctggagtgggtctcagctattagtggtagtggtggtagcacatactacgcagactccgtgaagggccggttcaccatctccagagacaattccaagaacacgctgtatctgcaaatgaacagcctgagagccgaggacacggccgtatattactgtgcgaaaaatcccatacagctatggtctaaaataaagaactggttcgacccctggggccagggaaccctggtcaccgtctcctcagggagtgcatccgccccaaagcttgaagaaggtgaattttcagaagcacgcgtacaggctgtggtgactcaagagccctcactaagtgtgtccccaggagggacagtcagtctcacctgtggctccagcgctggagatgtcacctatggtcactttccctactggtaccagcagaagcctggccaagcccccagaatgctcatttatgatgtaaacaacagagcgtcctggacccctgcccggttctcaggctccctcgttgggggcaaggctgccctgaccctttcgggtgcgcagcctggggatgaggctgactattactgcgccctctcctattttggttctatgtttttcggcggagggaccaagctgaccgtcctcagtcagcccaaggctgccccctcggtcactctgttcccaccctcctctgcggccgcaggttctgaacaaaagctgatctcagaagaagatctatcccatcatcaccatcatcat

SEQ ID NO: 108 - DNA, 924 bp, synthetic construct
  source 1..924: mol_type = other DNA
atgaaatacctattgcctacggcagccgctggcttgctgctgctggcagctcagccggccatggccgaggtgcagctggtgcagtctgggggaggcgtggtccagcctgggaggtccctgagactctcctgtgcagcctctggattcaccttcagtagctatggcatgcactgggtccgccaggctccaggcaaggggctggagtgggtggcagttatttcatatgatggaagtaataaatactatgcagactccgtgaagggccgattcaccatctccagagacaattccaagaacacgctgtatctgcaaatgaacagcctgagagctgaggacacggctgtgtattattgtgcgaaagatcttacccgaagtggttatccttcctactactttgactactggggccagggaaccctggtcaccgtctcctcagggagtgcatccgccccaaagcttgaagaaggtgaattttcagaagcacgcgtatcttctgagctgactcaggaccctgctgtgtctgtggccttgggacggacagtcaggatcacatgccaaggagacagcctcagaagctattatgcaagctggtaccagcagaagccaggacaggcccctgtacttgtcatctatggtaaaaacaaccggccctcagggatcccagaccgattctctggctccagctcaggaaacacagcttccttgaccatcactggggctcaggcggaagatgaggctgactattactgtaactcccgggacagcagtggtaacctagtattcggcggagggaccaagctgaccgtcctaggtcagcccaaggctgccccctcggtcactctgttcccgccctcctctgcggccgcaggttctgaacaaaagctgatctcagaagaagatctatcccatcatcaccatcatcat

SEQ ID NO: 109 - protein, 4 aa, synthetic construct
GGGS

SEQ ID NO: 110 - protein, 10 aa, synthetic construct
ETSGGGGSRL

SEQ ID NO: 111 - protein, 16 aa, synthetic construct
SGGGGSGGGGSGGGGS

SEQ ID NO: 112 - protein, 5 aa, synthetic construct
GGGGS

SEQ ID NO: 113 - protein, 6 aa, synthetic construct
GGGGGS

SEQ ID NO: 114 - protein, 7 aa, synthetic construct
GGGGGGS

SEQ ID NO: 115 - protein, 15 aa, synthetic construct
GGGGSGGGGSGGGGS

SEQ ID NO: 116 - protein, 5 aa, synthetic construct
GGGGG

SEQ ID NO: 117 - protein, 10 aa, synthetic construct
GGGGSGGGGS

SEQ ID NO: 118 - protein, 20 aa, synthetic construct
GGGGSGGGGSGGGGSGGGGS

SEQ ID NO: 119 - protein, 6 aa, synthetic construct
GGGGGG

SEQ ID NO: 120 - protein, 6 aa, synthetic construct
GGGGGG

SEQ ID NO: 121 - protein, 8 aa, synthetic construct
GGGGGGGG

SEQ ID NO: 122 - protein, 18 aa, synthetic construct
KESGSVSSEQLAQFRSLD

SEQ ID NO: 123 - protein, 14 aa, synthetic construct
EGKSSGSGSESKST

SEQ ID NO: 124 - protein, 12 aa, synthetic construct
GSAGSAAGSGEF

SEQ ID NO: 125 - protein, 16 aa, synthetic construct
SGGGGSAGSAAGSGEF

SEQ ID NO: 126 - protein, 16 aa, synthetic construct
SGGGLLLLLLLLGGGS

SEQ ID NO: 127 - protein, 16 aa, synthetic construct
SGGGAAAAAAAAGGGS

SEQ ID NO: 128 - protein, 24 aa, synthetic construct
SGGGAAAAAAAAAAAAAAAAGGGS

SEQ ID NO: 129 - protein, 24 aa, synthetic construct
SGALGGLALAGLLLAGLGLGAAGS

SEQ ID NO: 130 - protein, 14 aa, synthetic construct
SLSLSPGGGGGPAR

SEQ ID NO: 131 - protein, 25 aa, synthetic construct
SLSLSPGGGGGPARSLSLSPGGGGG

SEQ ID NO: 132 - protein, 6 aa, synthetic construct
GSSGSS

SEQ ID NO: 133 - protein, 7 aa, synthetic construct
GSSSSSS

SEQ ID NO: 134 - protein, 6 aa, synthetic construct
GGSSSS

SEQ ID NO: 135 - protein, 6 aa, synthetic construct
GSSSSS

SEQ ID NO: 136 - protein, 6 aa, synthetic construct
SGGGGS

SEQ ID NO: 137 - protein, 21 aa, Homo sapiens
IYIWAPLAGTCGVLLLSLVIT

SEQ ID NO: 138 - protein, 219 aa, Homo sapiens
PCPAPPVAGPSVFLFPPKPKDTLMIARTPEVTCVVVDVSHEDPEVKFNWYVDGVEVHNAKTKPREEQYNSTYRVVSVLTVLHQDWLNGKEYKCKVSNKALPAPIEKTISKAKGQPREPQVYTLPPSRDELTKNQVSLTCLVKGFYPSDIAVEWESNGQPENNYKTTPPVLDSDGSFFLYSKLTVDKSRWQQGNVFSCSVMHEALHNHYTQKSLSLSPGK

SEQ ID NO: 139 - protein, 81 aa, synthetic construct
FVPVFLPAKPTTTPAPRPPTPAPTIASQPLSLRPEASRPAAGGAVHTRGLDFADIYIWAPLAGTCGVLLLSLVITLYCNHR

SEQ ID NO: 140 - protein, 54 aa, synthetic construct
FVPVFLPAKPTTTPAPRPPTPAPTIASQPLSLRPEASRPAAGGAVHTRGLDFAD

SEQ ID NO: 141 - protein, 82 aa, synthetic construct
FVPVFLPAKPTTTPAPRPPTPAPTIASQPLSLRPEACRPAAGGAVHTRGLDFACDIYIWAPLAGTCGVLLLSLVITLYCNHR

SEQ ID NO: 142 - protein, 66 aa, Homo sapiens
IEVMYPPPYLDNEKSNGTIIHVKGKHLCPSPLFPGPSKPFWVLVVVGGVLACYSLLVTVAFIIFWV

SEQ ID NO: 143 - protein, 21 aa, synthetic construct
MALPVTALLLPLALLLHAAAP

SEQ ID NO: 144 - protein, 21 aa, synthetic construct
MALPVTALLLPLALLLHAARP

SEQ ID NO: 145 - protein, 112 aa, Homo sapiens
RVKFSRSADAPAYQQGQNQLYNELNLGRREEYDVLDKRRGRDPEMGGKPRRKNPQEGLYNELQKDKMAEAYSEIGMKGERRRGKGHDGLYQGLSTATKDTYDALHMQALPPR

SEQ ID NO: 146 - protein, 68 aa, synthetic construct
FWVLVVVGGVLACYSLLVTVAFIIFWVRSKRSRLLHSDYMNMTPRRPGPTRKHYQPYAPPRDFAAYRS

SEQ ID NO: 147 - protein, 43 aa, Homo sapiens
WVRSKRSRLLHSDYMNMTPRRPGPTRKHYQPYAPPRDFAAYRS

SEQ ID NO: 148 - protein, 42 aa, synthetic construct
ALYLLRRDQRLPPDAHKPPGGGSFRTPIQEEQADAHSTLAKI

SEQ ID NO: 149 - protein, 42 aa, synthetic construct
KRGRKKLLYIFKQPFMRPVQTTQEEDGCSCRFPEEEEGGCEL

SEQ ID NO: 150 - protein, 38 aa, synthetic construct
CWLTKKKYSSSVHDPNGEYMFMRAVNTAKKSRLTDVTL

SEQ ID NO: 151 - protein, 197 aa, synthetic construct
TYTYRHCWPHKPLVTADEAGMEALTPPPATHLSPLDSAHTLLAPPDSSEKICTVQLVGNSWTPGYPETQEALCPQVTWSWDQLPSRALGPAAAPTLSPESPAGSPAMMLQPGPQLYDVMDAVPARRWKEFVRTLGLREAEIEAVEVEIGRFRDQQYEMLKRWRQQQPAGLGAVYAALERMGLDGCVEDLRSRLQRGP

SEQ ID NO: 152 - protein, 286 aa, Homo sapiens
NCRNTGPWLKKVLKCNTPDPSKFFSQLSSEHGGDVQKWLSSPFPSSSFSPGGLAPEISPLEVLERDKVTQLLLQQDKVPEPASLSSNHSLTSCFTNQGYFFFHLPDALEIEACQVYFTYDPYSEEDPDEGVAGAPTGSSPQPLQPLSGEDDAYCTFPSRDDLLLFSPSLLGGPSPPSTAPGGSGAGEERMPPSLQERVPRDWDPQPLGPPTPGVPDLVDFQPPPELVLREAGEEVPDAGPREGVSFPWSRPPGQGEFRALNARLPLNTDAYLSLQELQGQDPTHLV

SEQ ID NO: 153 - protein, 94 aa, synthetic construct
NCRNTGPWLKKVLKCNTPDPSKFFSQLSSEHGGDVQKWLSSPFPSSSFSPGGLAPEISPLEVLERDKVTQLLPLNTDAYLSLQELQGQDPTHLV

SEQ ID NO: 154 - protein, 208 aa, synthetic construct
NCRNTGPWLKKVLKCNTPDPSKFFSQLSSEHGGDVQKWLSSPFPSSSFSPGGLAPEISPLEVLERDKVTQLLDAYCTFPSRDDLLLFSPSLLGGPSPPSTAPGGSGAGEERMPPSLQERVPRDWDPQPLGPPTPGVPDLVDFQPPPELVLREAGEEVPDAGPREGVSFPWSRPPGQGEFRALNARLPLNTDAYLSLQELQGQDPTHLV

SEQ ID NO: 155 - protein, 431 aa, Homo sapiens
MPNPRPGKPSAPSLALGPSPGASPSWRAAPKASDLLGARGPGGTFQGRDLRGGAHASSSSLNPMPPSQLQLPTLPLVMVAPSGARLGPLPHLQALLQDRPHFMHQLSTVDAHARTPVLQVHPLESPAMISLTPPTTATGVFSLKARPGLPPGINVASLEWVSREPALLCTFPNPSAPRKDSTLSAVPQSSYPLLANGVCKWPGCEKVFEEPEDFLKHCQADHLLDEKGRAQCLLQREMVQSLEQQLVLEKEKLSAMQAHLAGKMALTKASSVASSDKGSCCIVAAGSQGPVVPAWSGPREAPDSLFAVRRHLWGSHGNSTFPEFLHNMDYFKFHNMRPPFTYATLIRWAILEAPEKQRTLNEIYHWFTRMFAFFRNHPATWKNAIRHNLSLHKCFVRVESEKGAVWTVDELEFRKKRSQRPSRCSNPTPGP

SEQ ID NO: 156 - protein, 362 aa, synthetic construct
GGAHASSSSLNPMPPSQLQLPTLPLVMVAPSGARLGPLPHLQALLQDRPHFMHQLSTVDAHARTPVLQVHPLESPAMISLTPPTTATGVFSLKARPGLPPGINVASLEWVSREPALLCTFPNPSAPRKDSTLSAVPQSSYPLLANGVCKWPGCEKVFEEPEDFLKHCQADHLLDEKGRAQCLLQREMVQSLEQQLVLEKEKLSAMQAHLAGKMALTKASSVASSDKGSCCIVAAGSQGPVVPAWSGPREAPDSLFAVRRHLWGSHGNSTFPEFLHNMDYFKFHNMRPPFTYATLIRWAILEAPEKQRTLNEIYHWFTRMFAFFRNHPATWKNAIRHNLSLHKCFVRVESEKGAVWTVDELEF

SEQ ID NO: 157 - protein, 431 aa, synthetic construct
MPNPRPGKPSAPSLALGPSPGASPSWRAAPKASDLLGARGPGGTFQGRDLRGGAHASSSSLNPMPPSQLQLPTLPLVMVAPSGARLGPLPHLQALLQDRPHFMHQLSTVDAHARTPVLQVHPLESPAMISLTPPTTATGVFSLKARPGLPPGINVASLEWVSREPALLCTFPNPSAPRKDSTLSAVPQSSYPLLANGVCKWPGCEKVFEEPEDFLKHCQADHLLDEKGRAQCLLQREMVQSLEQQLVLEKEKLSAMQAHLAGKMALTKASSVASSDKGSCCIVAAGSQGPVVPAWSGPREAPDSLFAVRRHLWGSHGNSTFPEFLHNMDYFKFHNMRPPFTYATLIRWAILEAPEKQRTLNEIYHWFTRMFAFFRNHPATWKNAIRHNLSLHKCFVRVESEKGAVWTVDELEFRKKREQRPSRCSNPTPGP

SEQ ID NO: 158 - protein, 431 aa, synthetic construct
MPNPRPGKPSAPSLALGPSPGASPSWRAAPKASDLLGARGPGGTFQGRDLRGGAHASSSSLNPMPPSQLQLPTLPLVMVAPSGARLGPLPHLQALLQDRPHFMHQLSTVDAHARTPVLQVHPLESPAMISLTPPTTATGVFSLKARPGLPPGINVASLEWVSREPALLCTFPNPSAPRKDSTLSAVPQSSYPLLANGVCKWPGCEKVFEEPEDFLKHCQADHLLDEKGRAQCLLQREMVQSLEQQLVLEKEKLSAMQAHLAGKMALTKASSVASSDKGSCCIVAAGSQGPVVPAWSGPREAPDSLFAVRRHLWGSHGNSTFPEFLHNMDYFKFHNMRPPFTYATLIRWAILEAPEKQRTLNEIYHWFTRMFAFFRNHPATWKNAIRHNLSLHKCFVRVESEKGAVWTVDELEFRKKRSQRPARCSNPTPGP

SEQ ID NO: 159 - protein, 431 aa, synthetic construct
MPNPRPGKPSAPSLALGPSPGASPSWRAAPKASDLLGARGPGGTFQGRDLRGGAHASSSSLNPMPPSQLQLPTLPLVMVAPSGARLGPLPHLQALLQDRPHFMHQLSTVDAHARTPVLQVHPLESPAMISLTPPTTATGVFSLKARPGLPPGINVASLEWVSREPALLCTFPNPSAPRKDSTLSAVPQSSYPLLANGVCKWPGCEKVFEEPEDFLKHCQADHLLDEKGRAQCLLQREMVQSLEQQLVLEKEKLSAMQAHLAGKMALTKASSVASSDKGSCCIVAAGSQGPVVPAWSGPREAPDSLFAVRRHLWGSHGNSTFPEFLHNMDYFKFHNMRPPFTYATLIRWAILEAPEKQRTLNEIYHWFTRMFAFFRNHPATWKNAIRHNLSLHKCFVRVESEKGAVWTVDELEFRKKREQRPARCSNPTPGP

SEQ ID NO: 160 - protein, 441 aa, synthetic construct
MPNPRPGKPSAPSLALGPSPGASPSWRAAPKASDLLGARGPGGTFQGRDLRGGAHASSSSLNPMPPSQLQLPTLPLVMVAPSGARLGPLPHLQALLQDRPHFMHQLSTVDAHARTPVLQVHPLESPAMISLTPPTTATGVFSLKARPGLPPGINVASLEWVSREPALLCTFPNPSAPRKDSTLSAVPQSSYPLLANGVCKWPGCEKVFEEPEDFLKHCQADHLLDEKGRAQCLLQREMVQSLEQVEELSAMQAHLAGKMALTKASSVASSDKGSCCIVAAGSQGPVVPAWSGPREAPDSLFAVRRHLWGSHGNSTFPEFLHNMDYFKFHNMRPPFTYATLIRWAILEAPEKQRTLNEIYHWFTRMFAFFRNHPATWKNAIRHNLSLHKCFVRVESEKGAVWTVDELEFRKKRSQRPSRCSNPTPGPEGRGSLLTCGDVEEN

SEQ ID NO: 161 - DNA, 1296 bp, synthetic construct
  source 1..1296: mol_type = other DNA
atgcccaaccccaggcctggcaagccctcggccccttccttggcccttggcccatccccaggagcctcgcccagctggagggctgcacccaaagcctcagacctgctgggggcccggggcccagggggaaccttccagggccgagatcttcgaggcggggcccatgcctcctcttcttccttgaaccccatgccaccatcgcagctgcagctgcccacactgcccctagtcatggtggcaccctccggggcacggctgggccccttgccccacttacaggcactcctccaggacaggccacatttcatgcaccagctctcaacggtggatgcccacgcccggacccctgtgctgcaggtgcaccccctggagagcccagccatgatcagcctcacaccacccaccaccgccactggggtcttctccctcaaggcccggcctggcctcccacctgggatcaacgtggccagcctggaatgggtgtccagggagccggcactgctctgcaccttcccaaatcccagtgcacccaggaaggacagcaccctttcggctgtgccccagagctcctacccactgctggcaaatggtgtctgcaagtggcccggatgtgagaaggtcttcgaagagccagaggacttcctcaagcactgccaggcggaccatcttctggatgagaagggcagggcacaatgtctcctccagagagagatggtacagtctctggagcagcagctggtgctggagaaggagaagctgagtgccatgcaggcccacctggctgggaaaatggcactgaccaaggcttcatctgtggcatcatccgacaagggctcctgctgcatcgtagctgctggcagccaaggccctgtcgtcccagcctggtctggcccccgggaggcccctgacagcctgtttgctgtccggaggcacctgtggggtagccatggaaacagcacattcccagagttcctccacaacatggactacttcaagttccacaacatgcgaccccctttcacctacgccacgctcatccgctgggccatcctggaggctccagagaagcagcggacactcaatgagatctaccactggttcacacgcatgtttgccttcttcagaaaccatcctgccacctggaagaacgccatccgccacaacctgagtctgcacaagtgctttgtgcgggtggagagcgagaagggggctgtgtggaccgtggatgagctggagttccgcaagaaacggagccagaggcccagcaggtgttccaaccctacacctggcccctga

SEQ ID NO: 162 - DNA, 1352 bp, synthetic construct
  source 1..1352: mol_type = other DNA
gaattcgtcgacatgcccaaccccagacccggcaagccttctgccccttctctggccctgggaccatctcctggcgcctccccatcttggagagccgcccctaaagccagcgatctgctgggagctagaggccctggcggcacattccagggcagagatctgagaggcggagcccacgcctctagcagcagcctgaatcccatgccccctagccagctgcagctgcctacactgcctctcgtgatggtggcccctagcggagctagactgggccctctgcctcatctgcaggctctgctgcaggaccggccccactttatgcaccagctgagcaccgtggacgcccacgccagaacacctgtgctgcaggtgcaccccctggaaagccctgccatgatcagcctgacccctccaaccacagccaccggcgtgttcagcctgaaggccagacctggactgccccctggcatcaatgtggccagcctggaatgggtgtcccgcgaacctgccctgctgtgcaccttccccaatcctagcgcccccagaaaggacagcacactgtctgccgtgccccagagcagctatcccctgctggctaacggcgtgtgcaagtggcctggctgcgagaaggtgttcgaggaacccgaggacttcctgaagcactgccaggccgaccatctgctggacgagaaaggcagagcccagtgcctgctgcagcgcgagatggtgcagtccctggaacagcagctggtgctggaaaaagaaaagctgagcgccatgcaggcccacctggccggaaagatggccctgacaaaagccagcagcgtggccagctccgacaagggcagctgttgtatcgtggccgctggcagccagggacctgtggtgcctgcttggagcggacctagagaggcccccgatagcctgtttgccgtgcggagacacctgtggggcagccacggcaactctaccttccccgagttcctgcacaacatggactacttcaagttccacaacatgaggccccccttcacctacgccaccctgatcagatgggccattctggaagcccccgagaagcagcggaccctgaacgagatctaccactggtttacccggatgttcgccttcttccggaaccaccccgccacctggaagaacgccatccggcacaatctgagcctgcacaagtgcttcgtgcgggtggaaagcgagaagggcgccgtgtggacagtggacgagctggaatttcggaagaagcggtcccagaggcccagccggtgtagcaatcctacacctggccctgagggcagaggaagtctgctaacatgcggtgacgtcgaggagaatcc

SEQ ID NO: 163 - protein, 19 aa, synthetic construct
ATNFSLLKQAGDVEENPGP

SEQ ID NO: 164 - protein, 18 aa, synthetic construct
EGRGSLLTCGDVEENPGP

SEQ ID NO: 165 - protein, 20 aa, synthetic construct
QCTNYALLKLAGDVESNPGP

SEQ ID NO: 166 - protein, 22 aa, synthetic construct
VKQTLNFDLLKLAGDVESNPGP

SEQ ID NO: 167 - skipped

SEQ ID NO: 168 - protein, 4 aa, synthetic construct
RRKR

SEQ ID NO: 169 - DNA, 407 bp, synthetic construct
  source 1..407: mol_type = other DNA
gtaacgccattttgcaaggcatggaaaaataccaaaccaagaatagagaagttcagatcaagggcgggtacatgaaaatagctaacgttgggccaaacaggatatctgcggtgagcagtttcggccccggcccggggccaagaacagatggtcaccgcagtttcggccccggcccgaggccaagaacagatggtccccagatatggcccaaccctcagcagtttcttaagacccatcagatgtttccaggctcccccaaggacctgaaatgaccctgcgccttatttgaattaaccaatcagcctgcttctcgcttctgttcgcgcgcttctgcttcccgagctctataaaagagctcacaacccctcactcggcgcgccagtcctccgacagactgagtcggccgg

SEQ ID NO: 170 - protein, 530 aa, Homo sapiens
TEPLRPELRCNPGQFACRSGTIQCIPLPWQCDGWATCEDESDEANCPEVTGEVRPHHGKEAVDPRQGRARGGDPSHFHAVNVAQPVRFSSFLGKCPTGWHHYEGTASCYRVYLSGENYWDAAQTCQRLNGSLATFSTDQELRFVLAQEWDQPERSFGWKDQRKLWVGYQYVITGRNRSLEGRWEVAFKGSSEVFLPPDPIFASAMSENDNVFCAQLQCFHFPTLRHHDLHSWHAESCYEKSSFLCKRSQTCVDIKDNVVDEGFYFTPKGDDPCLSCTCHGGEPEMCVAALCERPQGCQQYRKDPKECCKFMCLDPDGNSLFDSMASGMRLVVSCISSFLILSLLLFMVHRLRQRRRERIESLIGANLHHFNLGRRIPGFDYGPDGFGTGLTPLHLSDDGEGGTFHFHDPPPPYTAYKYPDIGQPDDPPPPYEASIHPDSVFYDPADDDAFEPVEVSLPAPGDGGSEGALLRRLEQPLPTAGASLADLEDSADSSSALLVPPDPAQSGSTPAAEALPGGGRHSRSSLNTVV

SEQ ID NO: 171 - protein, 524 aa, Mus musculus
RPELRCNPGQFACHGGTIQCIPLPWQCDGWPTCEDKSDEADCPVTGEARPYGKETVDLRQGRARGGDPTHFHTVNVAQPVRFSSFLGKCPSGWHHYEGTASCYRVYLSGENYWDAAQTCQRVNGSLATFSTDQELRFVLAQEWDQPERSFGWKDQRKLWVGYQYVITGRNHSLEGRWEVAFKGSPEVFLPPDPIFASAMSENDNVFCAQLQCFHFPTLRHHDLHSWHAESCSEKSSFLCKRSQTCVDIKDNVVDEGFYFTPKGDDPCLSCTCHRGEPEMCVAALCERPQGCQQYRKDPKECCKFMCLDPDGSSLFDSMASGMRLVVSCISSFLILSLLLFMVHRLAQRRRERIESLIGANLHHFNLGRRIPGFDYGPDGFGTGLTPLHLSDDGEGGTFHFHDPPPPYTAYKYPDMDQPDDPPPPYEASINPDSVFYDPADDDAFEPVEASLPAPRDGGIEGALPRHLDQPLPPAETSLADLEDSTDSSSALLVPPDPAQSGSTPATEAPPGGGRLPRASLNTVV

SEQ ID NO: 172 - protein, 12 aa, synthetic construct
KLEEGEFSEARV

SEQ ID NO: 173 - protein, 12 aa, synthetic construct
ILEEGEFSEAGC

SEQ ID NO: 174 - protein, 12 aa, synthetic construct
  VARIANT 1: note = K or I
  VARIANT 11: note = R or G
  VARIANT 12: note = V or C
XLEEGEFSEAXX

SEQ ID NO: 175 - protein, 231 aa, synthetic construct
EPKSPDKTHTCPPCPAPPVAGPSVFLFPPKPKDTLMIARTPEVTCVVVDVSHEDPEVKFNWYVDGVEVHNAKTKPREEQYNSTYRVVSVLTVLHQDWLNGKEYKCKVSNKALPAPIEKTISKAKGQPREPQVYTLPPSRDELTKNQVSLTCLVKGFYPSDIAVEWESNGQPENNYKTTPPVLDSDGSFFLYSKLTVDKSRWQQGNVFSCSVMHEALHNHYTQKSLSLSPGK

SEQ ID NO: 176 - protein, 55 aa, Homo sapiens
FVPVFLPAKPTTTPAPRPPTPAPTIASQPLSLRPEACRPAAGGAVHTRGLDFACD

SEQ ID NO: 177 - protein, 22 aa, Homo sapiens
MALIVLGGVAGLLLFIGLGIFF

SEQ ID NO: 178 - protein, 494 aa, synthetic construct
QVQLVQSGGGVVQPGRSLRLSCAASGFTFSSYGMHWVRQAPGKGLEWVAVISYDGSNKYYADSVKGRFTISRDNSKNTLYLQMNSLRAEDTAVYYCAKDRGAVAGTDWYFDLWGRGTLVTVSSGGGGSGGGGSGGGGSSSELTQDPAVSVALGQTVRITCQGDSLRSYYASWYQQKPGQAPVLVIYGKNNRPSGIPDRFSGSSSGNTASLTITGAQAEDEADYYCNSRDSSGNHVVFGGGTKLTVLTRFVPVFLPAKPTTTPAPRPPTPAPTIASQPLSLRPEACRPAAGGAVHTRGLDFACDIYIWAPLAGTCGVLLLSLVITLYCNHRPPALEWVRSKRSRLLHSDYMNMTPRRPGPTRKHYQPYAPPRDFAAYRSASCTRVKFSRSADAPAYQQGQNQLYNELNLGRREEYDVLDKRRGRDPEMGGKPRRKNPQEGLYNELQKDKMAEAYSEIGMKGERRRGKGHDGLYQGLSTATKDTYDALHMQALPPR

SEQ ID NO: 179 - protein, 493 aa, synthetic construct
QVQLVQSGGGLVQPGGSLRLSCAASGFTFSSYSMSWVRQAPGKGLEWVLGITRGGNTFYADSVTGRFTISRDISKNTVFLQMDSLRVEDTAIYYCAKDWTMSGINVFDTWGQGTLVTVSSGGGGSGGGGSGGGGSQAVLTQPPSVSGSPGQSVTISCTGTSSDVGAYNRVSWYQQPPGTAPKLMIYEVNNRPSGVPDRFSGSKSGNTASLTISGLQAEDEADYYCSSSTTSSTYVFGTGTKVTVLTRFVPVFLPAKPTTTPAPRPPTPAPTIASQPLSLRPEACRPAAGGAVHTRGLDFACDIYIWAPLAGTCGVLLLSLVITLYCNHRPPALEWVRSKRSRLLHSDYMNMTPRRPGPTRKHYQPYAPPRDFAAYRSASCTRVKFSRSADAPAYQQGQNQLYNELNLGRREEYDVLDKRRGRDPEMGGKPRRKNPQEGLYNELQKDKMAEAYSEIGMKGERRRGKGHDGLYQGLSTATKDTYDALHMQALPPR

SEQ ID NO: 180 - protein, 487 aa, synthetic construct
EVQLQQSGGGLVQPGGSLRLSCAASEFPFSSYAMSWVRQAPGKGLAWVSAISSSGGDTYYADSVKGRFTISRDNSKNTLYLQMNSLRAEDTAVYYCAKNWNLDYWGQGTLVTVSSGGGGSGGGGSGGGGSSSELTQDPAVSVALGQTVMITCQGHSLRSYYASWYQQKPGQAPLLVIYGDNRRPSGIPDRFSGSNSGNTASLTITGTQAEDEADYYCNSRDSSGHHNVLFGGGTKLTVLTRFVPVFLPAKPTTTPAPRPPTPAPTIASQPLSLRPEACRPAAGGAVHTRGLDFACDIYIWAPLAGTCGVLLLSLVITLYCNHRPPALEWVRSKRSRLLHSDYMNMTPRRPGPTRKHYQPYAPPRDFAAYRSASCTRVKFSRSADAPAYQQGQNQLYNELNLGRREEYDVLDKRRGRDPEMGGKPRRKNPQEGLYNELQKDKMAEAYSEIGMKGERRRGKGHDGLYQGLSTATKDTYDALHMQALPPR

SEQ ID NO: 181 - protein, 484 aa, synthetic construct
EVQLVESGGGLVQPGGSLRLSCAASGFTVSSNYMSWVRQAPGKGLEWVSVIYSGGSTYYADSVKGRFTISRDNAKNSLYLQMNSLRAEDTAVYYCARGWTTFDYWGQGTLVTVSSGGGGSGGGGSGGGGSQAVLTQPPSLSVSPRQTVTITCSGDQLGDRYVSWYQQKPGQSPMLVIYQDDRRPSGVPERFSGSNSGNTATLTIGGTQAMDQADYYCQTWDNSPVVFGGGTKLTVLTRFVPVFLPAKPTTTPAPRPPTPAPTIASQPLSLRPEACRPAAGGAVHTRGLDFACDIYIWAPLAGTCGVLLLSLVITLYCNHRPPALEWVRSKRSRLLHSDYMNMTPRRPGPTRKHYQPYAPPRDFAAYRSASCTRVKFSRSADAPAYQQGQNQLYNELNLGRREEYDVLDKRRGRDPEMGGKPRRKNPQEGLYNELQKDKMAEAYSEIGMKGERRRGKGHDGLYQGLSTATKDTYDALHMQALPPR

SEQ ID NO: 182 - protein, 494 aa, synthetic construct
EVQLVQSGGGVVQPGRSLRLSCAASGFTFSSYGMHWVRQAPGKGLEWVAVISYDGSNKYYADSVKGRFTISRDNSKNTLYLQMNSLRAEDTAVYYCAKDLTRSGYPSYYFDYWGQGTLVTVSSGGGGSGGGGSGGGGSSSELTQDPAVSVALGQTVRITCQGDSLRSYYASWYQQKPGQAPVLVIYGKNNRPSGIPDRFSGSSSGNTASLTITGAQAEDEADYYCNSRGSSGNNWVFGGGTKLTVLTRFVPVFLPAKPTTTPAPRPPTPAPTIASQPLSLRPEACRPAAGGAVHTRGLDFACDIYIWAPLAGTCGVLLLSLVITLYCNHRPPALEWVRSKRSRLLHSDYMNMTPRRPGPTRKHYQPYAPPRDFAAYRSASCTRVKFSRSADAPAYQQGQNQLYNELNLGRREEYDVLDKRRGRDPEMGGKPRRKNPQEGLYNELQKDKMAEAYSEIGMKGERRRGKGHDGLYQGLSTATKDTYDALHMQALPPR

SEQ ID NO: 183 - protein, 488 aa, synthetic construct
QVQLVESGGGLVQPGGSLRLSCAASGFTFSSNAMSWVRQAPGKGLEWVSAIGTGGTTYYADSVKGRFTISRDNSKNTLYLQMNSLRAEDTAVYYCAKTGQLDYWGQGTLVTVSSGGGGSGGGGSGGGGSQSALTQPASVSGSPGQSITISCTGTSSDVGGYNYVSWFQQHPDKAPKLMIYDVSNRPSGVSNRFSGSKSGTSASLAISGLRSEDEADYYCAAWDDSLSGWVFGGGTKLTVLTRFVPVFLPAKPTTTPAPRPPTPAPTIASQPLSLRPEACRPAAGGAVHTRGLDFACDIYIWAPLAGTCGVLLLSLVITLYCNHRPPALEWVRSKRSRLLHSDYMNMTPRRPGPTRKHYQPYAPPRDFAAYRSASCTRVKFSRSADAPAYQQGQNQLYNELNLGRREEYDVLDKRRGRDPEMGGKPRRKNPQEGLYNELQKDKMAEAYSEIGMKGERRRGKGHDGLYQGLSTATKDTYDALHMQALPPR

SEQ ID NO: 184 - protein, 496 aa, synthetic construct
QVQLVQSGGGLVQPGGSLRLSCAASGFTFSNYAMSWVRQAPGKGLEWVSGISGGGDNTYYTDSVKGRFTISRDNSKNTLYLQMNSLTAEDTALYYCAKKQSGGSGWSLWGFDYWGQGTLVTVSSGGGGSGGGGSGGGGSQAVVTQEPSLTVSPGGTVTLTCASSTGAVTSGYYPSWFQQKPGQAPRPLIYNTNNKHSWSPARFSGSLLGGKAALTLSGVQPEDEADYYCLLYYGGRGVFGGGTRLTVLTRFVPVFLPAKPTTTPAPRPPTPAPTIASQPLSLRPEACRPAAGGAVHTRGLDFACDIYIWAPLAGTCGVLLLSLVITLYCNHRPPALEWVRSKRSRLLHSDYMNMTPRRPGPTRKHYQPYAPPRDFAAYRSASCTRVKFSRSADAPAYQQGQNQLYNELNLGRREEYDVLDKRRGRDPEMGGKPRRKNPQEGLYNELQKDKMAEAYSEIGMKGERRRGKGHDGLYQGLSTATKDTYDALHMQALPPR

SEQ ID NO: 185 - protein, 496 aa, synthetic construct
EVQLLESGGGLVQPGGSLRLSCAASGFTFSSYAMSWVRQAPGKGLEWVSAISGSGGSTYYADSVKGRFTISRDNSKNTLYLQMNSLRAEDTAVYYCAKNPIQLWSKIKNWFDPWGQGTLVTVSSGGGGSGGGGSGGGGSQAVVTQEPSLSVSPGGTVSLTCGSSAGDVTYGHFPYWYQQKPGQAPRMLIYDVNNRASWTPARFSGSLVGGKAALTLSGAQPGDEADYYCALSYFGSMFFGGGTKLTVLTRFVPVFLPAKPTTTPAPRPPTPAPTIASQPLSLRPEACRPAAGGAVHTRGLDFACDIYIWAPLAGTCGVLLLSLVITLYCNHRPPALEWVRSKRSRLLHSDYMNMTPRRPGPTRKHYQPYAPPRDFAAYRSASCTRVKFSRSADAPAYQQGQNQLYNELNLGRREEYDVLDKRRGRDPEMGGKPRRKNPQEGLYNELQKDKMAEAYSEIGMKGERRRGKGHDGLYQGLSTATKDTYDALHMQALPPR

SEQ ID NO: 186 - protein, 493 aa, synthetic construct
EVQLVQSGGGVVQPGRSLRLSCAASGFTFSSYGMHWVRQAPGKGLEWVAVISYDGSNKYYADSVKGRFTISRDNSKNTLYLQMNSLRAEDTAVYYCAKDLTRSGYPSYYFDYWGQGTLVTVSSGGGGSGGGGSGGGGSSSELTQDPAVSVALGRTVRITCQGDSLRSYYASWYQQKPGQAPVLVIYGKNNRPSGIPDRFSGSSSGNTASLTITGAQAEDEADYYCNSRDSSGNLVFGGGTKLTVLTRFVPVFLPAKPTTTPAPRPPTPAPTIASQPLSLRPEACRPAAGGAVHTRGLDFACDIYIWAPLAGTCGVLLLSLVITLYCNHRPPALEWVRSKRSRLLHSDYMNMTPRRPGPTRKHYQPYAPPRDFAAYRSASCTRVKFSRSADAPAYQQGQNQLYNELNLGRREEYDVLDKRRGRDPEMGGKPRRKNPQEGLYNELQKDKMAEAYSEIGMKGERRRGKGHDGLYQGLSTATKDTYDALHMQALPPR

SEQ ID NO: 187 - protein, 667 aa, synthetic construct
QVQLVQSGGGVVQPGRSLRLSCAASGFTFSSYGMHWVRQAPGKGLEWVAVISYDGSNKYYADSVKGRFTISRDNSKNTLYLQMNSLRAEDTAVYYCAKDRGAVAGTDWYFDLWGRGTLVTVSSGGGGSGGGGSGGGGSSSELTQDPAVSVALGQTVRITCQGDSLRSYYASWYQQKPGQAPVLVIYGKNNRPSGIPDRFSGSSSGNTASLTITGAQAEDEADYYCNSRDSSGNHVVFGGGTKLTVLTREPKSPDKTHTCPPCPAPPVAGPSVFLFPPKPKDTLMIARTPEVTCVVVDVSHEDPEVKFNWYVDGVEVHNAKTKPREEQYNSTYRVVSVLTVLHQDWLNGKEYKCKVSNKALPAPIEKTISKAKGQPREPQVYTLPPSRDELTKNQVSLTCLVKGFYPSDIAVEWESNGQPENNYKTTPPVLDSDGSFFLYSKLTVDKSRWQQGNVFSCSVMHEALHNHYTQKSLSLSPGKKDPKFWVLVVVGGVLACYSLLVTVAFIIFWVRSKRSRLLHSDYMNMTPRRPGPTRKHYQPYAPPRDFAAYRSASCTRVKFSRSADAPAYQQGQNQLYNELNLGRREEYDVLDKRRGRDPEMGGKPRRKNPQEGLYNELQKDKMAEAYSEIGMKGERRRGKGHDGLYQGLSTATKDTYDALHMQALPPR

SEQ ID NO: 188 - protein, 666 aa, synthetic construct
QVQLVQSGGGLVQPGGSLRLSCAASGFTFSSYSMSWVRQAPGKGLEWVLGITRGGNTFYADSVTGRFTISRDISKNTVFLQMDSLRVEDTAIYYCAKDWTMSGINVFDTWGQGTLVTVSSGGGGSGGGGSGGGGSQAVLTQPPSVSGSPGQSVTISCTGTSSDVGAYNRVSWYQQPPGTAPKLMIYEVNNRPSGVPDRFSGSKSGNTASLTISGLQAEDEADYYCSSSTTSSTYVFGTGTKVTVLTREPKSPDKTHTCPPCPAPPVAGPSVFLFPPKPKDTLMIARTPEVTCVVVDVSHEDPEVKFNWYVDGVEVHNAKTKPREEQYNSTYRVVSVLTVLHQDWLNGKEYKCKVSNKALPAPIEKTISKAKGQPREPQVYTLPPSRDELTKNQVSLTCLVKGFYPSDIAVEWESNGQPENNYKTTPPVLDSDGSFFLYSKLTVDKSRWQQGNVFSCSVMHEALHNHYTQKSLSLSPGKKDPKFWVLVVVGGVLACYSLLVTVAFIIFWVRSKRSRLLHSDYMNMTPRRPGPTRKHYQPYAPPRDFAAYRSASCTRVKFSRSADAPAYQQGQNQLYNELNLGRREEYDVLDKRRGRDPEMGGKPRRKNPQEGLYNELQKDKMAEAYSEIGMKGERRRGKGHDGLYQGLSTATKDTYDALHMQALPPR

SEQ ID NO: 189 - protein, 660 aa, synthetic construct
EVQLQQSGGGLVQPGGSLRLSCAASEFPFSSYAMSWVRQAPGKGLAWVSAISSSGGDTYYADSVKGRFTISRDNSKNTLYLQMNSLRAEDTAVYYCAKNWNLDYWGQGTLVTVSSGGGGSGGGGSGGGGSSSELTQDPAVSVALGQTVMITCQGHSLRSYYASWYQQKPGQAPLLVIYGDNRRPSGIPDRFSGSNSGNTASLTITGTQAEDEADYYCNSRDSSGHHNVLFGGGTKLTVLTREPKSPDKTHTCPPCPAPPVAGPSVFLFPPKPKDTLMIARTPEVTCVVVDVSHEDPEVKFNWYVDGVEVHNAKTKPREEQYNSTYRVVSVLTVLHQDWLNGKEYKCKVSNKALPAPIEKTISKAKGQPREPQVYTLPPSRDELTKNQVSLTCLVKGFYPSDIAVEWESNGQPENNYKTTPPVLDSDGSFFLYSKLTVDKSRWQQGNVFSCSVMHEALHNHYTQKSLSLSPGKKDPKFWVLVVVGGVLACYSLLVTVAFIIFWVRSKRSRLLHSDYMNMTPRRPGPTRKHYQPYAPPRDFAAYRSASCTRVKFSRSADAPAYQQGQNQLYNELNLGRREEYDVLDKRRGRDPEMGGKPRRKNPQEGLYNELQKDKMAEAYSEIGMKGERRRGKGHDGLYQGLSTATKDTYDALHMQALPPR

SEQ ID NO: 190 - protein, 657 aa, synthetic construct
EVQLVESGGGLVQPGGSLRLSCAASGFTVSSNYMSWVRQAPGKGLEWVSVIYSGGSTYYADSVKGRFTISRDNAKNSLYLQMNSLRAEDTAVYYCARGWTTFDYWGQGTLVTVSSGGGGSGGGGSGGGGSQAVLTQPPSLSVSPRQTVTITCSGDQLGDRYVSWYQQKPGQSPMLVIYQDDRRPSGVPERFSGSNSGNTATLTIGGTQAMDQADYYCQTWDNSPVVFGGGTKLTVLTREPKSPDKTHTCPPCPAPPVAGPSVFLFPPKPKDTLMIARTPEVTCVVVDVSHEDPEVKFNWYVDGVEVHNAKTKPREEQYNSTYRVVSVLTVLHQDWLNGKEYKCKVSNKALPAPIEKTISKAKGQPREPQVYTLPPSRDELTKNQVSLTCLVKGFYPSDIAVEWESNGQPENNYKTTPPVLDSDGSFFLYSKLTVDKSRWQQGNVFSCSVMHEALHNHYTQKSLSLSPGKKDPKFWVLVVVGGVLACYSLLVTVAFIIFWVRSKRSRLLHSDYMNMTPRRPGPTRKHYQPYAPPRDFAAYRSASCTRVKFSRSADAPAYQQGQNQLYNELNLGRREEYDVLDKRRGRDPEMGGKPRRKNPQEGLYNELQKDKMAEAYSEIGMKGERRRGKGHDGLYQGLSTATKDTYDALHMQALPPR

SEQ ID NO: 191 - protein, 667 aa, synthetic construct
EVQLVQSGGGVVQPGRSLRLSCAASGFTFSSYGMHWVRQAPGKGLEWVAVISYDGSNKYYADSVKGRFTISRDNSKNTLYLQMNSLRAEDTAVYYCAKDLTRSGYPSYYFDYWGQGTLVTVSSGGGGSGGGGSGGGGSSSELTQDPAVSVALGQTVRITCQGDSLRSYYASWYQQKPGQAPVLVIYGKNNRPSGIPDRFSGSSSGNTASLTITGAQAEDEADYYCNSRGSSGNNWVFGGGTKLTVLTREPKSPDKTHTCPPCPAPPVAGPSVFLFPPKPKDTLMIARTPEVTCVVVDVSHEDPEVKFNWYVDGVEVHNAKTKPREEQYNSTYRVVSVLTVLHQDWLNGKEYKCKVSNKALPAPIEKTISKAKGQPREPQVYTLPPSRDELTKNQVSLTCLVKGFYPSDIAVEWESNGQPENNYKTTPPVLDSDGSFFLYSKLTVDKSRWQQGNVFSCSVMHEALHNHYTQKSLSLSPGKKDPKFWVLVVVGGVLACYSLLVTVAFIIFWVRSKRSRLLHSDYMNMTPRRPGPTRKHYQPYAPPRDFAAYRSASCTRVKFSRSADAPAYQQGQNQLYNELNLGRREEYDVLDKRRGRDPEMGGKPRRKNPQEGLYNELQKDKMAEAYSEIGMKGERRRGKGHDGLYQGLSTATKDTYDALHMQALPPR

SEQ ID NO: 192 - protein, 661 aa, synthetic construct
QVQLVESGGGLVQPGGSLRLSCAASGFTFSSNAMSWVRQAPGKGLEWVSAIGTGGTTYYADSVKGRFTISRDNSKNTLYLQMNSLRAEDTAVYYCAKTGQLDYWGQGTLVTVSSGGGGSGGGGSGGGGSQSALTQPASVSGSPGQSITISCTGTSSDVGGYNYVSWFQQHPDKAPKLMIYDVSNRPSGVSNRFSGSKSGTSASLAISGLRSEDEADYYCAAWDDSLSGWVFGGGTKLTVLTREPKSPDKTHTCPPCPAPPVAGPSVFLFPPKPKDTLMIARTPEVTCVVVDVSHEDPEVKFNWYVDGVEVHNAKTKPREEQYNSTYRVVSVLTVLHQDWLNGKEYKCKVSNKALPAPIEKTISKAKGQPREPQVYTLPPSRDELTKNQVSLTCLVKGFYPSDIAVEWESNGQPENNYKTTPPVLDSDGSFFLYSKLTVDKSRWQQGNVFSCSVMHEALHNHYTQKSLSLSPGKKDPKFWVLVVVGGVLACYSLLVTVAFIIFWVRSKRSRLLHSDYMNMTPRRPGPTRKHYQPYAPPRDFAAYRSASCTRVKFSRSADAPAYQQGQNQLYNELNLGRREEYDVLDKRRGRDPEMGGKPRRKNPQEGLYNELQKDKMAEAYSEIGMKGERRRGKGHDGLYQGLSTATKDTYDALHMQALPPR

SEQ ID NO: 193 - protein, 669 aa, synthetic construct
QVQLVQSGGGLVQPGGSLRLSCAASGFTFSNYAMSWVRQAPGKGLEWVSGISGGGDNTYYTDSVKGRFTISRDNSKNTLYLQMNSLTAEDTALYYCAKKQSGGSGWSLWGFDYWGQGTLVTVSSGGGGSGGGGSGGGGSQAVVTQEPSLTVSPGGTVTLTCASSTGAVTSGYYPSWFQQKPGQAPRPLIYNTNNKHSWSPARFSGSLLGGKAALTLSGVQPEDEADYYCLLYYGGRGVFGGGTRLTVLTREPKSPDKTHTCPPCPAPPVAGPSVFLFPPKPKDTLMIARTPEVTCVVVDVSHEDPEVKFNWYVDGVEVHNAKTKPREEQYNSTYRVVSVLTVLHQDWLNGKEYKCKVSNKALPAPIEKTISKAKGQPREPQVYTLPPSRDELTKNQVSLTCLVKGFYPSDIAVEWESNGQPENNYKTTPPVLDSDGSFFLYSKLTVDKSRWQQGNVFSCSVMHEALHNHYTQKSLSLSPGKKDPKFWVLVVVGGVLACYSLLVTVAFIIFWVRSKRSRLLHSDYMNMTPRRPGPTRKHYQPYAPPRDFAAYRSASCTRVKFSRSADAPAYQQGQNQLYNELNLGRREEYDVLDKRRGRDPEMGGKPRRKNPQEGLYNELQKDKMAEAYSEIGMKGERRRGKGHDGLYQGLSTATKDTYDALHMQALPPR

SEQ ID NO: 194 - protein, 669 aa, synthetic construct
EVQLLESGGGLVQPGGSLRLSCAASGFTFSSYAMSWVRQAPGKGLEWVSAISGSGGSTYYADSVKGRFTISRDNSKNTLYLQMNSLRAEDTAVYYCAKNPIQLWSKIKNWFDPWGQGTLVTVSSGGGGSGGGGSGGGGSQAVVTQEPSLSVSPGGTVSLTCGSSAGDVTYGHFPYWYQQKPGQAPRMLIYDVNNRASWTPARFSGSLVGGKAALTLSGAQPGDEADYYCALSYFGSMFFGGGTKLTVLTREPKSPDKTHTCPPCPAPPVAGPSVFLFPPKPKDTLMIARTPEVTCVVVDVSHEDPEVKFNWYVDGVEVHNAKTKPREEQYNSTYRVVSVLTVLHQDWLNGKEYKCKVSNKALPAPIEKTISKAKGQPREPQVYTLPPSRDELTKNQVSLTCLVKGFYPSDIAVEWESNGQPENNYKTTPPVLDSDGSFFLYSKLTVDKSRWQQGNVFSCSVMHEALHNHYTQKSLSLSPGKKDPKFWVLVVVGGVLACYSLLVTVAFIIFWVRSKRSRLLHSDYMNMTPRRPGPTRKHYQPYAPPRDFAAYRSASCTRVKFSRSADAPAYQQGQNQLYNELNLGRREEYDVLDKRRGRDPEMGGKPRRKNPQEGLYNELQKDKMAEAYSEIGMKGERRRGKGHDGLYQGLSTATKDTYDALHMQALPPR

SEQ ID NO: 195 - protein, 666 aa, synthetic construct
EVQLVQSGGGVVQPGRSLRLSCAASGFTFSSYGMHWVRQAPGKGLEWVAVISYDGSNKYYADSVKGRFTISRDNSKNTLYLQMNSLRAEDTAVYYCAKDLTRSGYPSYYFDYWGQGTLVTVSSGGGGSGGGGSGGGGSSSELTQDPAVSVALGRTVRITCQGDSLRSYYASWYQQKPGQAPVLVIYGKNNRPSGIPDRFSGSSSGNTASLTITGAQAEDEADYYCNSRDSSGNLVFGGGTKLTVLTREPKSPDKTHTCPPCPAPPVAGPSVFLFPPKPKDTLMIARTPEVTCVVVDVSHEDPEVKFNWYVDGVEVHNAKTKPREEQYNSTYRVVSVLTVLHQDWLNGKEYKCKVSNKALPAPIEKTISKAKGQPREPQVYTLPPSRDELTKNQVSLTCLVKGFYPSDIAVEWESNGQPENNYKTTPPVLDSDGSFFLYSKLTVDKSRWQQGNVFSCSVMHEALHNHYTQKSLSLSPGKKDPKFWVLVVVGGVLACYSLLVTVAFIIFWVRSKRSRLLHSDYMNMTPRRPGPTRKHYQPYAPPRDFAAYRSASCTRVKFSRSADAPAYQQGQNQLYNELNLGRREEYDVLDKRRGRDPEMGGKPRRKNPQEGLYNELQKDKMAEAYSEIGMKGERRRGKGHDGLYQGLSTATKDTYDALHMQALPPR

SEQ ID NO: 196 - protein, 58 aa, synthetic construct
FSSVVPVLQKVNSTTTKPVLRTPSPVHPTGTSQPQRPEDCRPRGSVKGTGLDFACDIY

SEQ ID NO: 197 - DNA, 174 bp, synthetic construct
  source 1..174: mol_type = other DNA
ttcagctctgtggtgcccgtgctgcagaaagtgaacagcaccaccacaaagcctgtgctgagaaccccttctcctgtgcaccctaccggcacaagccagcctcaaagacctgaggactgcagacctagaggctccgtgaaaggcacaggcctggacttcgcctgcgacatctat

SEQ ID NO: 198 - protein, 8 aa, synthetic construct
  VARIANT 8: note = G or S or A
GFTFSSYX

SEQ ID NO: 199 - protein, 8 aa, synthetic construct
  VARIANT 6: note = N or S
GFTFSXYA

SEQ ID NO: 200 - protein, 8 aa, synthetic construct
  VARIANT 7: note = N or Y
GFTFSSXA

SEQ ID NO: 201 - protein, 9 aa, synthetic construct
  VARIANT 6: note = A or G
  VARIANT 9: note = R or Y
SSDVGXYNX

SEQ ID NO: 202-204 - skipped (3 entries)

SEQ ID NO: 205 - protein, 10 aa, synthetic construct
  VARIANT 9: note = H or L
NSRDSSGNXV

SEQ ID NO: 206 - protein, 11 aa, synthetic construct
  VARIANT 8: note = N or H
  VARIANT 10: note = N or V
NSRDSSGXHXV